European Patent Specification EP 3 681 995 B1, published July 16, 2025. Title: CELL. Applicant: Autolus Limited. The sequence listing filed with the application follows.

SEQUENCE LISTING (14 sequences)

SEQ ID NO: 1 - protein, 29 aa, Artificial Sequence
  first dimerization domain sequence
QLEKELQALEKENAQLEWELQALEKELAQ

SEQ ID NO: 2 - protein, 29 aa, Artificial Sequence
  second dimerization domain sequence
QLEKKLQALKKKNAQLKWKLQALKKKLAQ

SEQ ID NO: 3 - protein, 4 aa, Artificial Sequence
  linker sequence
GGSG

SEQ ID NO: 4 - protein, 6 aa, Artificial Sequence
  linker sequence
GSGSGS

SEQ ID NO: 5 - protein, 8 aa, Artificial Sequence
  linker sequence
GGSGGGSG

SEQ ID NO: 6 - protein, 9 aa, Artificial Sequence
  linker sequence
SGGSGGSGG

SEQ ID NO: 7 - protein, 1590 aa, Artificial Sequence
  constitutively active Signal Transducer and Activator of Transcription (STAT) construct (STAT3 - Linker - STAT5)
MAQWNQLQQLDTRYLEQLHQLYSDSFPMELRQFLAPWIESQDWAYAASKESHATLVFHNLLGEIDQQYSRFLQESNVLYQHNLRRIKQFLQSRYLEKPMEIARIVARCLWEESRLLQTAATAAQQGGQANHPTAAVVTEKQQMLEQHLQDVRKRVQDLEQKMKVVENLQDDFDFNYKTLKSQGDMQDLNGNNQSVTRQKMQQLEQMLTALDQMRRSIVSELAGLLSAMEYVQKTLTDEELADWKRRQQIACIGGPPNICLDRLENWITSLAESQLQTRQQIKKLEELQQKVSYKGDPIVQHRPMLEERIVELFRNLMKSAFVVERQPCMPMHPDRPLVIKTGVQFTTKVRLLVKFPELNYQLKIKVCIDKDSGDVAALRGSRKFNILGTNTKVMNMEESNNGSLSAEFKHLTLREQRCGNGGRANCDASLIVTEELHLITFETEVYHQGLKIDLETHSLPVVVISNICQMPNAWASILWYNMLTNNPKNVNFFTKPPIGTWDQVAEVLSWQFSSTTKRGLSIEQLTTLAEKLLGPGVNYSGCQITWAKFCKENMAGKGFSFWVWLDNIIDLVKKYILALWNEGYIMGFISKERERAILSTKPPGTFLLRFSESSKEGGVTFTWVEKDISGKTQIQSVEPYTKQQLNNMSFAEIIMGYKIMDATNILVSPLVYLYPDIPKEEAFGKYCRPESQEHPEADPGSAAPYLKTKFICVTPTTCSNTIDLPMSPRTLDSLMQFGNNGEGAEPSAGGQFESLTFDMELTSECATSPMSGGGGSGGGGSGGGGSGGGGSGGGGSMAGWIQAQQLQGDALRQMQVLYGQHFPIEVRHYLAQWIESQPWDAIDLDNPQDRAQATQLLEGLVQELQKKAEHQVGEDGFLLKIKLGHYATQLQKTYDRCPLELVRCIRHILYNEQRLVREANNCSSPAGILVDAMSQKHLQINQTFEELRLVTQDTENELKKLQQTQEYFIIQYQESLRIQAQFAQLAQLSPQERLSRETALQQKQVSLEAWLQREAQTLQQYRVELAEKHQKTLQLLRKQQTIILDDELIQWKRRQQLAGNGGPPEGSLDVLQSWCEKLAEIIWQNRQQIRRAEHLCQQLPIPGPVEEMLAEVNATITDIISALVTSTFIIEKQPPQVLKTQTKFAATVRLLVGGKLNVHMNPPQVKATIISEQQAKSLLKNENTRNECSGEILNNCCVMEYHQATGTLSAHFRNMSLKRIKRADRRGAESVTEEKFTVLFESQFSVGSNELVFQVKTLSLPVVVIVHGSQDHNATATVLWDNAFAEPGRVPFAVPDKVLWPQLCEALNMKFKAEVQSNRGLTKENLVFLAQKLFNNSSSHLEDYSGLSVSWSQFNRENLPGWNYTFWQWFDGVMEVLKKHHKPHWNDGAILGFVNKQQAHDLLINKPDGTFLLRFSDSEIGGITIAWKFDSPERNLWNLKPFTTRDFSIRSLADRLGDLSYLIYVFPDRPKDEVFSKYYTPVLAKAVDGYVKPQIKQVVPEFVNASADAGGSSATYMDQAPSPAVCPQAPYNMYPQNPDHVLDQDGEFDLDETMDVARHVEELLRRPMDSLDSRLSPPAGLFTSARGSLS

SEQ ID NO: 8 - protein, 1896 aa, Artificial Sequence
  constitutively active STAT construct (TIP - STAT3 - Linker - STAT5 - 2a - Myristoylation and palmitoylation sequence - Ridge Linker - TetRB)
MWTWNAYAFAAPSGGGSAQWNQLQQLDTRYLEQLHQLYSDSFPMELRQFLAPWIESQDWAYAASKESHATLVFHNLLGEIDQQYSRFLQESNVLYQHNLRRIKQFLQSRYLEKPMEIARIVARCLWEESRLLQTAATAAQQGGQANHPTAAVVTEKQQMLEQHLQDVRKRVQDLEQKMKVVENLQDDFDFNYKTLKSQGDMQDLNGNNQSVTRQKMQQLEQMLTALDQMRRSIVSELAGLLSAMEYVQKTLTDEELADWKRRQQIACIGGPPNICLDRLENWITSLAESQLQTRQQIKKLEELQQKVSYKGDPIVQHRPMLEERIVELFRNLMKSAFVVERQPCMPMHPDRPLVIKTGVQFTTKVRLLVKFPELNYQLKIKVCIDKDSGDVAALRGSRKFNILGTNTKVMNMEESNNGSLSAEFKHLTLREQRCGNGGRANCDASLIVTEELHLITFETEVYHQGLKIDLETHSLPVVVISNICQMPNAWASILWYNMLTNNPKNVNFFTKPPIGTWDQVAEVLSWQFSSTTKRGLSIEQLTTLAEKLLGPGVNYSGCQITWAKFCKENMAGKGFSFWVWLDNIIDLVKKYILALWNEGYIMGFISKERERAILSTKPPGTFLLRFSESSKEGGVTFTWVEKDISGKTQIQSVEPYTKQQLNNMSFAEIIMGYKIMDATNILVSPLVYLYPDIPKEEAFGKYCRPESQEHPEADPGSAAPYLKTKFICVTPTTCSNTIDLPMSPRTLDSLMQFGNNGEGAEPSAGGQFESLTFDMELTSECATSPMSGGGGSGGGGSGGGGSGGGGSGGGGSMAGWIQAQQLQGDALRQMQVLYGQHFPIEVRHYLAQWIESQPWDAIDLDNPQDRAQATQLLEGLVQELQKKAEHQVGEDGFLLKIKLGHYATQLQKTYDRCPLELVRCIRHILYNEQRLVREANNCSSPAGILVDAMSQKHLQINQTFEELRLVTQDTENELKKLQQTQEYFIIQYQESLRIQAQFAQLAQLSPQERLSRETALQQKQVSLEAWLQREAQTLQQYRVELAEKHQKTLQLLRKQQTIILDDELIQWKRRQQLAGNGGPPEGSLDVLQSWCEKLAEIIWQNRQQIRRAEHLCQQLPIPGPVEEMLAEVNATITDIISALVTSTFIIEKQPPQVLKTQTKFAATVRLLVGGKLNVHMNPPQVKATIISEQQAKSLLKNENTRNECSGEILNNCCVMEYHQATGTLSAHFRNMSLKRIKRADRRGAESVTEEKFTVLFESQFSVGSNELVFQVKTLSLPVVVIVHGSQDHNATATVLWDNAFAEPGRVPFAVPDKVLWPQLCEALNMKFKAEVQSNRGLTKENLVFLAQKLFNNSSSHLEDYSGLSVSWSQFNRENLPGWNYTFWQWFDGVMEVLKKHHKPHWNDGAILGFVNKQQAHDLLINKPDGTFLLRFSDSEIGGITIAWKFDSPERNLWNLKPFTTRDFSIRSLADRLGDLSYLIYVFPDRPKDEVFSKYYTPVLAKAVDGYVKPQIKQVVPEFVNASADAGGSSATYMDQAPSPAVCPQAPYNMYPQNPDHVLDQDGEFDLDETMDVARHVEELLRRPMDSLDSRLSPPAGLFTSARGSLSEGRGSLLTCGDVEENPGPMGCGCSSHPELEAEAAAKEAAAKEAAAKEAAAKALEAEAAAKEAAAKEAAAKEAAAKALESGGGSMSRLDKSKVINSALELLNEVGIEGLTTRKLAQKLGVEQPTLYWHVKNKRALLDALAIEMLDRHHTHFCPLEGESWQDFLRNNAKSFRCALLSHRDGAKVHLGTRPTEKQYETLENQLAFLCQQGFSLENALYALSAVGHFTLGCVLEDQEHQVAKEERETPTTDSMPPLLRQAIELFDHQGAEPAFLFGLELIICGLEKQLKCESGS

SEQ ID NO: 9 - protein, 2729 aa, Artificial Sequence
  constitutively active STAT construct (SH2 ZAP70 - Linker - TEV - 2a - myristoylation and palmitoylation sequence - linker - TEV cleavage site x3 - STAT3 - Linker -STAT5 - 2a - aCD19)
MPDPAAHLPFFYGSISRAEAEEHLKLAGMADGLFLLRQCLRSLGGYVLSLVHDVRFHHFPIERQLNGTYAIAGGKAHCGPAELCEFYSRDPDGLPCNLRKPCNRPSGLEPQPGVFDCLRDAMVRDYVRQTWKLEGEALEQAIISQAPQVEKLIATTAHERMPWYHSSLTREEAERKLYSGAQTDGKFLLRPRKEQGTYALSLIYGKTVYHYLISQDKAGKYCIPEGTKFDTLWQLVEYLKLKADGLIYCLKEACPNSSASNASGAAAPTLPAHPSTLTHPSGGGGSSLFKGPRDYNPISSTICHLTNESDGHTTSLYGIGFGPFIITNKHLFRRNNGTLLVQSLHGVFKVKNTTTLQQHLIDGRDMIIIRMPKDFPPFPQKLKFREPQREERICLVTTNFQTKSMSSMVSDTSCTFPSSDGIFWKHWIQTKDGQCGSPLVSTRDGFIVGIHSASNFTNTNNYFTSVPKNFMELLTNQEAQQWVSGWRLNADSVLWGGHKVFMSKPEEPFQPVKEATQLMNELVYSQEGRGSLLTCGDVEENPGPMGCGCSSHPESGGGGSGGGGSENLYFQGENLYFQGENLYFQGENLYFQGENLYFQGENLYFQGENLYFQGENLYFQGENLYFQGAQWNQLQQLDTRYLEQLHQLYSDSFPMELRQFLAPWIESQDWAYAASKESHATLVFHNLLGEIDQQYSRFLQESNVLYQHNLRRIKQFLQSRYLEKPMEIARIVARCLWEESRLLQTAATAAQQGGQANHPTAAVVTEKQQMLEQHLQDVRKRVQDLEQKMKVVENLQDDFDFNYKTLKSQGDMQDLNGNNQSVTRQKMQQLEQMLTALDQMRRSIVSELAGLLSAMEYVQKTLTDEELADWKRRQQIACIGGPPNICLDRLENWITSLAESQLQTRQQIKKLEELQQKVSYKGDPIVQHRPMLEERIVELFRNLMKSAFVVERQPCMPMHPDRPLVIKTGVQFTTKVRLLVKFPELNYQLKIKVCIDKDSGDVAALRGSRKFNILGTNTKVMNMEESNNGSLSAEFKHLTLREQRCGNGGRANCDASLIVTEELHLITFETEVYHQGLKIDLETHSLPVVVISNICQMPNAWASILWYNMLTNNPKNVNFFTKPPIGTWDQVAEVLSWQFSSTTKRGLSIEQLTTLAEKLLGPGVNYSGCQITWAKFCKENMAGKGFSFWVWLDNIIDLVKKYILALWNEGYIMGFISKERERAILSTKPPGTFLLRFSESSKEGGVTFTWVEKDISGKTQIQSVEPYTKQQLNNMSFAEIIMGYKIMDATNILVSPLVYLYPDIPKEEAFGKYCRPESQEHPEADPGSAAPYLKTKFICVTPTTCSNTIDLPMSPRTLDSLMQFGNNGEGAEPSAGGQFESLTFDMELTSECATSPMSGGGGSGGGGSGGGGSGGGGSGGGGSMAGWIQAQQLQGDALRQMQVLYGQHFPIEVRHYLAQWIESQPWDAIDLDNPQDRAQATQLLEGLVQELQKKAEHQVGEDGFLLKIKLGHYATQLQKTYDRCPLELVRCIRHILYNEQRLVREANNCSSPAGILVDAMSQKHLQINQTFEELRLVTQDTENELKKLQQTQEYFIIQYQESLRIQAQFAQLAQLSPQERLSRETALQQKQVSLEAWLQREAQTLQQYRVELAEKHQKTLQLLRKQQTIILDDELIQWKRRQQLAGNGGPPEGSLDVLQSWCEKLAEIIWQNRQQIRRAEHLCQQLPIPGPVEEMLAEVNATITDIISALVTSTFIIEKQPPQVLKTQTKFAATVRLLVGGKLNVHMNPPQVKATIISEQQAKSLLKNENTRNECSGEILNNCCVMEYHQATGTLSAHFRNMSLKRIKRADRRGAESVTEEKFTVLFESQFSVGSNELVFQVKTLSLPVVVIVHGSQDHNATATVLWDNAFAEPGRVPFAVPDKVLWPQLCEALNMKFKAEVQSNRGLTKENLVFLAQKLFNNSSSHLEDYSGLSVSWSQFNRENLPGWNYTFWQWFDGVMEVLKKHHKPHWNDGAILGFVNKQQAHDLLINKPDGTFLLRFSDSEIGGITIAWKFDSPERNLWNLKPFTTRDFSIRSLADRLGDLSYLIYVFPDRPKDEVFSKYYTPVLAKAVDGYVKPQIKQVVPEFVNASADAGGSSATYMDQAPSPAVCPQAPYNMYPQNPDHVLDQDGEFDLDETMDVARHVEELLRRPMDSLDSRLSPPAGLFTSARGSLSEGRGSLLTCGDVEENPGPMETDTLLLWVLLLWVPGSTGDIQMTQTTSSLSASLGDRVTISCRASQDISKYLNWYQQKPDGTVKLLIYHTSRLHSGVPSRFSGSGSGTDYSLTISNLEQEDIATYFCQQGNTLPYTFGGGTKLEITKAGGGGSGGGGSGGGGSGGGGSEVKLQESGPGLVAPSQSLSVTCTVSGVSLPDYGVSWIRQPPRKGLEWLGVIWGSETTYYNSALKSRLTIIKDNSKSQVFLKMNSLQTDDTAIYYCAKHYYYGGSYAMDYWGQGTSVTVSSDPTTTPAPRPPTPAPTIASQPLSLRPEACRPAAGGAVHTRGLDFACDIYIWAPLAGTCGVLLLSLVITLYCKRGRKKLLYIFKQPFMRPVQTTQEEDGCSCRFPEEEEGGCELRVKFSRSADAPAYQQGQNQLYNELNLGRREEYDVLDKRRGRDPEMGGKPRRKNPQEGLYNELQKDKMAEAYSEIGMKGERRRGKGHDGLYQGLSTATKDTYDALHMQALPPR

SEQ ID NO: 10 - protein, 2430 aa, Artificial Sequence
  constitutively active STAT construct (TIP - Linker - dZap70SH2 - linker - TEV - 2a - Truncated CD22 - CD19TM - Tyro-1 endodomain - Linker - TetRB - 2A - aCD19 - linker - TEV cleavage site x 3 - GOFSTAT5(S710F)
MWTWNAYAFAAPSGGGSMPDPAAHLPFFYGSISRAEAEEHLKLAGMADGLFLLRQCLRSLGGYVLSLVHDVRFHHFPIERQLNGTYAIAGGKAHCGPAELCEFYSRDPDGLPCNLRKPCNRPSGLEPQPGVFDCLRDAMVRDYVRQTWKLEGEALEQAIISQAPQVEKLIATTAHERMPWYHSSLTREEAERKLYSGAQTDGKFLLRPRKEQGTYALSLIYGKTVYHYLISQDKAGKYCIPEGTKFDTLWQLVEYLKLKADGLIYCLKEACPNSSASNASGAAAPTLPAHPSTLTHPSGGGGSSLFKGPRDYNPISSTICHLTNESDGHTTSLYGIGFGPFIITNKHLFRRNNGTLLVQSLHGVFKVKNTTTLQQHLIDGRDMIIIRMPKDFPPFPQKLKFREPQREERICLVTTNFQTKSMSSMVSDTSCTFPSSDGIFWKHWIQTKDGQCGSPLVSTRDGFIVGIHSASNFTNTNNYFTSVPKNFMELLTNQEAQQWVSGWRLNADSVLWGGHKVFMSKPEEPFQPVKEATQLMNELVYSQEGRGSLLTCGDVEENPGPMETDTLLLWVLLLWVPGSTGDSSGKPIPNPLLGLDSSGGGSAPRDVRVRKIKPLSEIHSGNSVSLQCDFSSSHPKEVQFFWEKNGRLLGKESQLNFDSISPEDAGSYSCWVNNSIGQTASKAWTLEVLYAPRRLRVSMSPGDQVMEGKSATLTCESDANPPVSHYTWFDWNNQSLPYHSQKLRLEPVKVQHSGAYWCQGTNSVGKGRSPLSTLTVYYSPETIGRRAVTLAYLIFCLCSLVGILHLRARRSMDEANQPLLTDQYQCYAEEYEKLQNPNQSVVGGSGGSMSRLDKSKVINSALELLNEVGIEGLTTRKLAQKLGVEQPTLYWHVKNKRALLDALAIEMLDRHHTHFCPLEGESWQDFLRNNAKSFRCALLSHRDGAKVHLGTRPTEKQYETLENQLAFLCQQGFSLENALYALSAVGHFTLGCVLEDQEHQVAKEERETPTTDSMPPLLRQAIELFDHQGAEPAFLFGLELIICGLEKQLKCESGSEGRGSLLTCGDVEENPGPMETDTLLLWVLLLWVPGSTGDIQMTQTTSSLSASLGDRVTISCRASQDISKYLNWYQQKPDGTVKLLIYHTSRLHSGVPSRFSGSGSGTDYSLTISNLEQEDIATYFCQQGNTLPYTFGGGTKLEITKAGGGGSGGGGSGGGGSGGGGSEVKLQESGPGLVAPSQSLSVTCTVSGVSLPDYGVSWIRQPPRKGLEWLGVIWGSETTYYNSALKSRLTIIKDNSKSQVFLKMNSLQTDDTAIYYCAKHYYYGGSYAMDYWGQGTSVTVSSDPTTTPAPRPPTPAPTIASQPLSLRPEACRPAAGGAVHTRGLDFACDIYIWAPLAGTCGVLLLSLVITLYCKRGRKKLLYIFKQPFMRPVQTTQEEDGCSCRFPEEEEGGCELRVKFSRSADAPAYQQGQNQLYNELNLGRREEYDVLDKRRGRDPEMGGKPRRKNPQEGLYNELQKDKMAEAYSEIGMKGERRRGKGHDGLYQGLSTATKDTYDALHMQALPPRGGSGGSENLYFQGENLYFQGENLYFQGENLYFQGENLYFQGENLYFQGENLYFQGENLYFQGENLYFQGMAGWIQAQQLQGDALRQMQVLYGQHFPIEVRHYLAQWIESQPWDAIDLDNPQDRAQATQLLEGLVQELQKKAEHQVGEDGFLLKIKLGHYATQLQKTYDRCPLELVRCIRHILYNEQRLVREANNCSSPAGILVDAMSQKHLQINQTFEELRLVTQDTENELKKLQQTQEYFIIQYQESLRIQAQFAQLAQLSPQERLSRETALQQKQVSLEAWLQREAQTLQQYRVELAEKHQKTLQLLRKQQTIILDDELIQWKRRQQLAGNGGPPEGSLDVLQSWCEKLAEIIWQNRQQIRRAEHLCQQLPIPGPVEEMLAEVNATITDIISALVTSTFIIEKQPPQVLKTQTKFAATVRLLVGGKLNVHMNPPQVKATIISEQQAKSLLKNENTRNECSGEILNNCCVMEYHQATGTLSAHFRNMSLKRIKRADRRGAESVTEEKFTVLFESQFSVGSNELVFQVKTLSLPVVVIVHGSQDHNATATVLWDNAFAEPGRVPFAVPDKVLWPQLCEALNMKFKAEVQSNRGLTKENLVFLAQKLFNNSSSHLEDYSGLSVSWSQFNRENLPGWNYTFWQWFDGVMEVLKKHHKPHWNDGAILGFVNKQQAHDLLINKPDGTFLLRFSDSEIGGITIAWKFDSPERNLWNLKPFTTRDFSIRSLADRLGDLSYLIYVFPDRPKDEVFSKYYTPVLAKAVDGYVKPQIKQVVPEFVNAFADAGGSSATYMDQAPSPAVCPQAPYNMYPQNPDHVLDQDGEFDLDETMDVARHVEELLRRPMDSLDSRLSPPAGLFTSARGSLS

SEQ ID NO: 11 - protein, 1813 aa, Artificial Sequence
  constitutively active STAT construct (FRB - linker - STAT5 - 2a - FKBP12 - linker - STAT3)
ILWHEMWHEGLEEASRLYFGERNVKGMFEVLEPLHAMMERGPQTLKETSFNQAYGRDLMEAQEWCRKYMKSGNVKDLLQAWDLYYHVFRRISKSGGGGSGGGGSGGGGSMAGWIQAQQLQGDALRQMQVLYGQHFPIEVRHYLAQWIESQPWDAIDLDNPQDRAQATQLLEGLVQELQKKAEHQVGEDGFLLKIKLGHYATQLQKTYDRCPLELVRCIRHILYNEQRLVREANNCSSPAGILVDAMSQKHLQINQTFEELRLVTQDTENELKKLQQTQEYFIIQYQESLRIQAQFAQLAQLSPQERLSRETALQQKQVSLEAWLQREAQTLQQYRVELAEKHQKTLQLLRKQQTIILDDELIQWKRRQQLAGNGGPPEGSLDVLQSWCEKLAEIIWQNRQQIRRAEHLCQQLPIPGPVEEMLAEVNATITDIISALVTSTFIIEKQPPQVLKTQTKFAATVRLLVGGKLNVHMNPPQVKATIISEQQAKSLLKNENTRNECSGEILNNCCVMEYHQATGTLSAHFRNMSLKRIKRADRRGAESVTEEKFTVLFESQFSVGSNELVFQVKTLSLPVVVIVHGSQDHNATATVLWDNAFAEPGRVPFAVPDKVLWPQLCEALNMKFKAEVQSNRGLTKENLVFLAQKLFNNSSSHLEDYSGLSVSWSQFNRENLPGWNYTFWQWFDGVMEVLKKHHKPHWNDGAILGFVNKQQAHDLLINKPDGTFLLRFSDSEIGGITIAWKFDSPERNLWNLKPFTTRDFSIRSLADRLGDLSYLIYVFPDRPKDEVFSKYYTPVLAKAVDGYVKPQIKQVVPEFVNASADAGGSSATYMDQAPSPAVCPQAPYNMYPQNPDHVLDQDGEFDLDETMDVARHVEELLRRPMDSLDSRLSPPAGLFTSARGSLSEGRGSLLTCGDVEENPGPGVQVETISPGDGRTFPKRGQTCVVHYTGMLEDGKKVDSSRDRNKPFKFMLGKQEVIRGWEEGVAQMSVGQRAKLTISPDYAYGATGHPGIIPPHATLVFDVELLKLESGGGGSGGGGSGGGGSAQWNQLQQLDTRYLEQLHQLYSDSFPMELRQFLAPWIESQDWAYAASKESHATLVFHNLLGEIDQQYSRFLQESNVLYQHNLRRIKQFLQSRYLEKPMEIARIVARCLWEESRLLQTAATAAQQGGQANHPTAAVVTEKQQMLEQHLQDVRKRVQDLEQKMKVVENLQDDFDFNYKTLKSQGDMQDLNGNNQSVTRQKMQQLEQMLTALDQMRRSIVSELAGLLSAMEYVQKTLTDEELADWKRRQQIACIGGPPNICLDRLENWITSLAESQLQTRQQIKKLEELQQKVSYKGDPIVQHRPMLEERIVELFRNLMKSAFVVERQPCMPMHPDRPLVIKTGVQFTTKVRLLVKFPELNYQLKIKVCIDKDSGDVAALRGSRKFNILGTNTKVMNMEESNNGSLSAEFKHLTLREQRCGNGGRANCDASLIVTEELHLITFETEVYHQGLKIDLETHSLPVVVISNICQMPNAWASILWYNMLTNNPKNVNFFTKPPIGTWDQVAEVLSWQFSSTTKRGLSIEQLTTLAEKLLGPGVNYSGCQITWAKFCKENMAGKGFSFWVWLDNIIDLVKKYILALWNEGYIMGFISKERERAILSTKPPGTFLLRFSESSKEGGVTFTWVEKDISGKTQIQSVEPYTKQQLNNMSFAEIIMGYKIMDATNILVSPLVYLYPDIPKEEAFGKYCRPESQEHPEADPGSAAPYLKTKFICVTPTTCSNTIDLPMSPRTLDSLMQFGNNGEGAEPSAGGQFESLTFDMELTSECATSPM

SEQ ID NO: 12 - protein, 1832 aa, Artificial Sequence
  constitutively active STAT construct (TIP - linker - STAT5 - 2a - TetRB - linker - STAT3)
MWTWNAYAFAAPSGGGGSGGGGSGGGGSMAGWIQAQQLQGDALRQMQVLYGQHFPIEVRHYLAQWIESQPWDAIDLDNPQDRAQATQLLEGLVQELQKKAEHQVGEDGFLLKIKLGHYATQLQKTYDRCPLELVRCIRHILYNEQRLVREANNCSSPAGILVDAMSQKHLQINQTFEELRLVTQDTENELKKLQQTQEYFIIQYQESLRIQAQFAQLAQLSPQERLSRETALQQKQVSLEAWLQREAQTLQQYRVELAEKHQKTLQLLRKQQTIILDDELIQWKRRQQLAGNGGPPEGSLDVLQSWCEKLAEIIWQNRQQIRRAEHLCQQLPIPGPVEEMLAEVNATITDIISALVTSTFIIEKQPPQVLKTQTKFAATVRLLVGGKLNVHMNPPQVKATIISEQQAKSLLKNENTRNECSGEILNNCCVMEYHQATGTLSAHFRNMSLKRIKRADRRGAESVTEEKFTVLFESQFSVGSNELVFQVKTLSLPVVVIVHGSQDHNATATVLWDNAFAEPGRVPFAVPDKVLWPQLCEALNMKFKAEVQSNRGLTKENLVFLAQKLFNNSSSHLEDYSGLSVSWSQFNRENLPGWNYTFWQWFDGVMEVLKKHHKPHWNDGAILGFVNKQQAHDLLINKPDGTFLLRFSDSEIGGITIAWKFDSPERNLWNLKPFTTRDFSIRSLADRLGDLSYLIYVFPDRPKDEVFSKYYTPVLAKAVDGYVKPQIKQVVPEFVNASADAGGSSATYMDQAPSPAVCPQAPYNMYPQNPDHVLDQDGEFDLDETMDVARHVEELLRRPMDSLDSRLSPPAGLFTSARGSLSEGRGSLLTCGDVEENPGPMSRLDKSKVINSALELLNEVGIEGLTTRKLAQKLGVEQPTLYWHVKNKRALLDALAIEMLDRHHTHFCPLEGESWQDFLRNNAKSFRCALLSHRDGAKVHLGTRPTEKQYETLENQLAFLCQQGFSLENALYALSAVGHFTLGCVLEDQEHQVAKEERETPTTDSMPPLLRQAIELFDHQGAEPAFLFGLELIICGLEKQLKCESGSSGGGGSGGGGSGGGGSAQWNQLQQLDTRYLEQLHQLYSDSFPMELRQFLAPWIESQDWAYAASKESHATLVFHNLLGEIDQQYSRFLQESNVLYQHNLRRIKQFLQSRYLEKPMEIARIVARCLWEESRLLQTAATAAQQGGQANHPTAAVVTEKQQMLEQHLQDVRKRVQDLEQKMKVVENLQDDFDFNYKTLKSQGDMQDLNGNNQSVTRQKMQQLEQMLTALDQMRRSIVSELAGLLSAMEYVQKTLTDEELADWKRRQQIACIGGPPNICLDRLENWITSLAESQLQTRQQIKKLEELQQKVSYKGDPIVQHRPMLEERIVELFRNLMKSAFVVERQPCMPMHPDRPLVIKTGVQFTTKVRLLVKFPELNYQLKIKVCIDKDSGDVAALRGSRKFNILGTNTKVMNMEESNNGSLSAEFKHLTLREQRCGNGGRANCDASLIVTEELHLITFETEVYHQGLKIDLETHSLPVVVISNICQMPNAWASILWYNMLTNNPKNVNFFTKPPIGTWDQVAEVLSWQFSSTTKRGLSIEQLTTLAEKLLGPGVNYSGCQITWAKFCKENMAGKGFSFWVWLDNIIDLVKKYILALWNEGYIMGFISKERERAILSTKPPGTFLLRFSESSKEGGVTFTWVEKDISGKTQIQSVEPYTKQQLNNMSFAEIIMGYKIMDATNILVSPLVYLYPDIPKEEAFGKYCRPESQEHPEADPGSAAPYLKTKFICVTPTTCSNTIDLPMSPRTLDSLMQFGNNGEGAEPSAGGQFESLTFDMELTSECATSPM

SEQ ID NO: 13 - protein, 4 aa, Artificial Sequence
  basic amino acid furin target sequence
  misc_feature (2)..(2): Xaa can be any naturally occurring amino acid
  MISC_FEATURE (3)..(3): Xaa may be Arg or Lys
RXXR

SEQ ID NO: 14 - protein, 7 aa, Artificial Sequence
  consensus Tobacco Etch Virus (TEV) cleavage site
ENLYFQS